European Patent Specification EP 3 708 587 B1, published May 22, 2024. Title: GENETICALLY MODIFIED CELLS AND USES THEREOF. Applicant: Cartherics Pty. Ltd. The sequence listing filed with the application follows.

SEQUENCE LISTING (25 sequences)

SEQ ID NO: 1 - DNA, 2670 bp, Artificial Sequence
  DNA coding for TAG72 CAR-P2A-CD47 binding receptor
atggagttcggcctgcgctgggtgttcctggtggccatcctgaaggacgtgcagtgccaggtgcagctgcagcagagcgacgccgagctggtgaagcccggcgccagcgtgaagatcagctgcaaggccagcggctacaccttcaccgaccacgccatccactgggtgaagcagaaccccgagcagggcctggagtggatcggctacttcagccccggcaacgacgacttcaagtacaacgagcgcttcaagggcaaggccaccctgaccgccgacaagagcagcagcaccgcctacctgcagctgaacagcctgaccagcgaggacagcgccgtgtacttctgcacccgcagcctgaacatggcctactggggccagggcaccagcgtgaccgtgagcagcggcggcggcggcagcggcggcggcggcagcggcggcggcggcagcgacatcgtgatgacccagagccccagcagcctgcccgtgagcgtgggcgagaaggtgaccctgagctgcaagagcagccagagcctgctgtacagcggcaaccagaagaactacctggcctggtaccagcagaagcccggccagagccccaagctcctgatctactgggccagcacccgcgagagcggcgtgcccgaccgcttcaccggcagcggcagcggcaccgacttcaccctgagcatcagcagcgtggagaccgaggacctggccgtgtactactgccagcagtactacagctaccccctgaccttcggcgccggcaccaagctggtgctgaagcgcgactacaaggacgacgacgacaagctgagcaactccatcatgtacttcagccacttcgtgccggtcttcctgccagcgaagcccaccacgacgccagcgccgcgaccaccaacaccggcgcccaccatcgcgtcgcagcccctgtccctgcgcccagaggcgtgccggccagcggcggggggcgcagtgcacacgagggggctgttttgggtgctggtggtggttggtggagtcctggcttgctatagcttgctagtaacagtggcctttattattttctgggtgaggagtaagaggagcaggctcctgcacagtgactacatgaacatgactccccgccgccccgggcccacccgcaagcattaccagccctatgccccaccacgcgacttcgcagcctatcgctccagagtgaagttcagcaggagcgcagacgcccccgcgtaccagcagggccagaaccagctctataacgagctcaatctaggacgaagagaggagtacgatgttttggacaagagacgtggccgggaccctgagatggggggaaagccgagaaggaagaaccctcaggaaggcctgtacaatgaactgcagaaagataagatggcggaggcctacagtgagattgggatgaaaggcgagcgccggaggggcaaggggcacgatggcctttaccagggtctcagtacagccaccaaggacacctacgacgcccttcacatgcaggccctgccccctcgcgtcgacggaagcggagctactaacttcagcctgctgaagcaggctggagacgtggaggagaaccctggacctatggccctgcccgtgaccgccctgctgctgcccctggccctgctgctgcacgccgcccgcgcccaggtgcagctggtgcagagcggcgccgaggtgaagaagcccggcgccagcgtgaaggtgagctgcaaggccagcggctacaccttcaccaactacaacatgcactgggtgcgccaggcccccggccagcgcctggagtggatgggcaccatctaccccggcaacgacgacaccagctacaaccagaagttcaaggaccgcgtgaccatcaccgccgacaccagcgccagcaccgcctacatggagctgagcagcctgcgcagcgaggacaccgccgtgtactactgcgcccgcggcggctaccgcgccatggactactggggccagggcaccctggtgaccgtgagcagcggcggaggcggaagcggaggcggaggcagcgggggcggcggaagcgacatcgtgatgacccagagccccctgagcctgcccgtgacccccggcgagcccgccagcatcagctgccgcagcagccagagcatcgtgtacagcaacggcaacacctacctgggctggtacctgcagaagcccggccagagcccccagctgctgatctacaaggtgagcaaccgcttcagcggcgtgcccgaccgcttcagcggcagcggcagcggcaccgacttcaccctgaagatcagccgcgtggaggccgaggacgtgggcgtgtactactgcttccagggcagccacgtgccctacaccttcggccagggcaccaagctggagatcaaggccgccgagcagaagctgatcagcgaggaggacctgatcgaggtgatgtacccccccccctacctggacaacgagaagagcaacggcaccatcatccacgtgaagggcaagcacctgtgccccagccccctgttccccggccccagcaagcccttctgggtgctggtggtggtgggcggcgtgctggcctgctacagcctgctggtgaccgtggccttcatcatcttctgggtgcgcagcaagcgcagccgcctgctgcacagcgactaa

SEQ ID NO: 2 - protein, 889 aa, Artificial Sequence
  Protein sequence of TAG72 CAR-P2A-CD47 binding receptor
  misc_feature (1)..(19): Kappa leader
  misc_feature (20)..(134): anti-TAG72 VH
  misc_feature (135)..(149): GS Linker
  misc_feature (150)..(263): anti-TAG72 VL
  misc_feature (264)..(272): FLAG epitope
  misc_feature (273)..(331): CD8 hinge
  misc_feature (332)..(358): CD28 TM
  misc_feature (359)..(399): CD28 Signalling domain
  misc_feature (400)..(513): TCR3-zeta Signalling domain
  misc_feature (514)..(535): P2A self cleaving peptide
  misc_feature (536)..(556): CD8a leader
  misc_feature (557)..(673): anti-CD47 VH
  misc_feature (674)..(688): GS linker
  misc_feature (689)..(800): anti-CD47 VL
  misc_feature (801)..(812): c-Myc epitope
  misc_feature (813)..(851): CD28 hinge
  misc_feature (852)..(878): CD28 TM
  misc_feature (879)..(889): cytoplasmic tail derived from CD28
MEFGLRWVFLVAILKDVQCQVQLQQSDAELVKPGASVKISCKASGYTFTDHAIHWVKQNPEQGLEWIGYFSPGNDDFKYNERFKGKATLTADKSSSTAYLQLNSLTSEDSAVYFCTRSLNMAYWGQGTSVTVSSGGGGSGGGGSGGGGSDIVMTQSPSSLPVSVGEKVTLSCKSSQSLLYSGNQKNYLAWYQQKPGQSPKLLIYWASTRESGVPDRFTGSGSGTDFTLSISSVETEDLAVYYCQQYYSYPLTFGAGTKLVLKRDYKDDDDKLSNSIMYFSHFVPVFLPAKPTTTPAPRPPTPAPTIASQPLSLRPEACRPAAGGAVHTRGLFWVLVVVGGVLACYSLLVTVAFIIFWVRSKRSRLLHSDYMNMTPRRPGPTRKHYQPYAPPRDFAAYRSRVKFSRSADAPAYQQGQNQLYNELNLGRREEYDVLDKRRGRDPEMGGKPRRKNPQEGLYNELQKDKMAEAYSEIGMKGERRRGKGHDGLYQGLSTATKDTYDALHMQALPPRVDGSGATNFSLLKQAGDVEENPGPMALPVTALLLPLALLLHAARAQVQLVQSGAEVKKPGASVKVSCKASGYTFTNYNMHWVRQAPGQRLEWMGTIYPGNDDTSYNQKFKDRVTITADTSASTAYMELSSLRSEDTAVYYCARGGYRAMDYWGQGTLVTVSSGGGGSGGGGSGGGGSDIVMTQSPLSLPVTPGEPASISCRSSQSIVYSNGNTYLGWYLQKPGQSPQLLIYKVSNRFSGVPDRFSGSGSGTDFTLKISRVEAEDVGVYYCFQGSHVPYTFGQGTKLEIKAAEQKLISEEDLIEVMYPPPYLDNEKSNGTIIHVKGKHLCPSPLFPGPSKPFWVLVVVGGVLACYSLLVTVAFIIFWVRSKRSRLLHSD

SEQ ID NO: 3 - DNA, 1062 bp, Artificial Sequence
  DNA coding for CD47-binding receptor
atggccctgcccgtgaccgccctgctgctgcccctggccctgctgctgcacgccgcccgcgcccaggtgcagctggtgcagagcggcgccgaggtgaagaagcccggcgccagcgtgaaggtgagctgcaaggccagcggctacaccttcaccaactacaacatgcactgggtgcgccaggcccccggccagcgcctggagtggatgggcaccatctaccccggcaacgacgacaccagctacaaccagaagttcaaggaccgcgtgaccatcaccgccgacaccagcgccagcaccgcctacatggagctgagcagcctgcgcagcgaggacaccgccgtgtactactgcgcccgcggcggctaccgcgccatggactactggggccagggcaccctggtgaccgtgagcagcggcggaggcggaagcggaggcggaggcagcgggggcggcggaagcgacatcgtgatgacccagagccccctgagcctgcccgtgacccccggcgagcccgccagcatcagctgccgcagcagccagagcatcgtgtacagcaacggcaacacctacctgggctggtacctgcagaagcccggccagagcccccagctgctgatctacaaggtgagcaaccgcttcagcggcgtgcccgaccgcttcagcggcagcggcagcggcaccgacttcaccctgaagatcagccgcgtggaggccgaggacgtgggcgtgtactactgcttccagggcagccacgtgccctacaccttcggccagggcaccaagctggagatcaaggccgccgagcagaagctgatcagcgaggaggacctgatcgaggtgatgtacccccccccctacctggacaacgagaagagcaacggcaccatcatccacgtgaagggcaagcacctgtgccccagccccctgttccccggccccagcaagcccttctgggtgctggtggtggtgggcggcgtgctggcctgctacagcctgctggtgaccgtggccttcatcatcttctgggtgcgcagcaagcgcagccgcctgctgcacagcgac

SEQ ID NO: 4 - protein, 354 aa, Artificial Sequence
  Protein sequence of CD47-binding receptor
  misc_feature (1)..(21): CD8a leader
  misc_feature (22)..(138): anti-CD47 VH
  misc_feature (139)..(153): GS linker
  misc_feature (154)..(265): anti-CD47 VL
  misc_feature (266)..(277): c-Myc epitope
  misc_feature (278)..(316): CD28 hinge
  misc_feature (317)..(343): CD28 TM
  misc_feature (344)..(354): cytoplasmic tail derived from CD28
MALPVTALLLPLALLLHAARAQVQLVQSGAEVKKPGASVKVSCKASGYTFTNYNMHWVRQAPGQRLEWMGTIYPGNDDTSYNQKFKDRVTITADTSASTAYMELSSLRSEDTAVYYCARGGYRAMDYWGQGTLVTVSSGGGGSGGGGSGGGGSDIVMTQSPLSLPVTPGEPASISCRSSQSIVYSNGNTYLGWYLQKPGQSPQLLIYKVSNRFSGVPDRFSGSGSGTDFTLKISRVEAEDVGVYYCFQGSHVPYTFGQGTKLEIKAAEQKLISEEDLIEVMYPPPYLDNEKSNGTIIHVKGKHLCPSPLFPGPSKPFWVLVVVGGVLACYSLLVTVAFIIFWVRSKRSRLLHSD

SEQ ID NO: 5 - DNA, 1065 bp, Artificial Sequence
  DNA coding for CD47-binding receptor with C to S substitution
atggccctgcccgtgaccgccctgctgctgcccctggccctgctgctgcacgccgcccgcgcccaggtgcagctggtgcagagcggcgccgaggtgaagaagcccggcgccagcgtgaaggtgagctgcaaggccagcggctacaccttcaccaactacaacatgcactgggtgcgccaggcccccggccagcgcctggagtggatgggcaccatctaccccggcaacgacgacaccagctacaaccagaagttcaaggaccgcgtgaccatcaccgccgacaccagcgccagcaccgcctacatggagctgagcagcctgcgcagcgaggacaccgccgtgtactactgcgcccgcggcggctaccgcgccatggactactggggccagggcaccctggtgaccgtgagcagcggcggaggcggaagcggaggcggaggcagcgggggcggcggaagcgacatcgtgatgacccagagccccctgagcctgcccgtgacccccggcgagcccgccagcatcagctgccgcagcagccagagcatcgtgtacagcaacggcaacacctacctgggctggtacctgcagaagcccggccagagcccccagctgctgatctacaaggtgagcaaccgcttcagcggcgtgcccgaccgcttcagcggcagcggcagcggcaccgacttcaccctgaagatcagccgcgtggaggccgaggacgtgggcgtgtactactgcttccagggcagccacgtgccctacaccttcggccagggcaccaagctggagatcaaggccgccgagcagaagctgatcagcgaggaggacctgatcgaggtgatgtacccccccccctacctggacaacgagaagagcaacggcaccatcatccacgtgaagggcaagcacctgagccccagccccctgttccccggccccagcaagcccttctgggtgctggtggtggtgggcggcgtgctggccagctacagcctgctggtgaccgtggccttcatcatcttctgggtgcgcagcaagcgcagccgcctgctgcacagcgactaa

SEQ ID NO: 6 - protein, 354 aa, Artificial Sequence
  Protein sequence of CD47-binding receptor with C to S substitution
MALPVTALLLPLALLLHAARAQVQLVQSGAEVKKPGASVKVSCKASGYTFTNYNMHWVRQAPGQRLEWMGTIYPGNDDTSYNQKFKDRVTITADTSASTAYMELSSLRSEDTAVYYCARGGYRAMDYWGQGTLVTVSSGGGGSGGGGSGGGGSDIVMTQSPLSLPVTPGEPASISCRSSQSIVYSNGNTYLGWYLQKPGQSPQLLIYKVSNRFSGVPDRFSGSGSGTDFTLKISRVEAEDVGVYYCFQGSHVPYTFGQGTKLEIKAAEQKLISEEDLIEVMYPPPYLDNEKSNGTIIHVKGKHLSPSPLFPGPSKPFWVLVVVGGVLASYSLLVTVAFIIFWVRSKRSRLLHSD

SEQ ID NO: 7 - DNA, 732 bp, Artificial Sequence
  DNA coding for TAG72 scFV
caggtgcagctgcagcagagcgacgccgagctggtgaagcccggcgccagcgtgaagatcagctgcaaggccagcggctacaccttcaccgaccacgccatccactgggtgaagcagaaccccgagcagggcctggagtggatcggctacttcagccccggcaacgacgacttcaagtacaacgagcgcttcaagggcaaggccaccctgaccgccgacaagagcagcagcaccgcctacctgcagctgaacagcctgaccagcgaggacagcgccgtgtacttctgcacccgcagcctgaacatggcctactggggccagggcaccagcgtgaccgtgagcagcggcggcggcggcagcggcggcggcggcagcggcggcggcggcagcgacatcgtgatgacccagagccccagcagcctgcccgtgagcgtgggcgagaaggtgaccctgagctgcaagagcagccagagcctgctgtacagcggcaaccagaagaactacctggcctggtaccagcagaagcccggccagagccccaagctcctgatctactgggccagcacccgcgagagcggcgtgcccgaccgcttcaccggcagcggcagcggcaccgacttcaccctgagcatcagcagcgtggagaccgaggacctggccgtgtactactgccagcagtactacagctaccccctgaccttcggcgccggcaccaagctggtgctgaagcgc

SEQ ID NO: 8 - protein, 244 aa, Artificial Sequence
  Protein sequence of TAG72 scFV
QVQLQQSDAELVKPGASVKISCKASGYTFTDHAIHWVKQNPEQGLEWIGYFSPGNDDFKYNERFKGKATLTADKSSSTAYLQLNSLTSEDSAVYFCTRSLNMAYWGQGTSVTVSSGGGGSGGGGSGGGGSDIVMTQSPSSLPVSVGEKVTLSCKSSQSLLYSGNQKNYLAWYQQKPGQSPKLLIYWASTRESGVPDRFTGSGSGTDFTLSISSVETEDLAVYYCQQYYSYPLTFGAGTKLVLKR

SEQ ID NO: 9 - protein, 117 aa, Artificial Sequence
  Protein sequence of Hu5F9 VH-2 (CD47)
QVQLVQSGAEVKKPGASVKVSCKASGYTFTNYNMHWVRQAPGQRLEWMGTIYPGNDDTSYNQKFKDRVTITADTSASTAYMELSSLRSEDTAVYYCARGGYRAMDYWGQGTLVTVSS

SEQ ID NO: 10 - protein, 112 aa, Artificial Sequence
  Protein sequence of Hu5F9 VL-12
DIVMTQSPLSLPVTPGEPASISCRSSQSIVYSNGNTYLGWYLQKPGQSPQLLIYKVSNRFSGVPDRFSGSGSGTDFTLKISRVEAEDVGVYYCFQGSHVPYTFGQGTKLEIK

SEQ ID NO: 11 - protein, 244 aa, Artificial Sequence
  Protein sequence of scFv for CD47 Attachment stalk
QVQLVQSGAEVKKPGASVKVSCKASGYTFTNYNMHWVRQAPGQRLEWMGTIYPGNDDTSYNQKFKDRVTITADTSASTAYMELSSLRSEDTAVYYCARGGYRAMDYWGQGTLVTVSSGGGGSGGGGSGGGGSDIVMTQSPLSLPVTPGEPASISCRSSQSIVYSNGNTYLGWYLQKPGQSPQLLIYKVSNRFSGVPDRFSGSGSGTDFTLKISRVEAEDVGVYYCFQGSHVPYTFGQGTKLEIK

SEQ ID NO: 12 - protein, 60 aa, Artificial Sequence
  CD8 hinge protein sequence
LSNSIMYFSHFVPVFLPAKPTTTPAPRPPTPAPTIASQPLSLRPEACRPAAGGAVHTRGL

SEQ ID NO: 13 - protein, 24 aa, Artificial Sequence
  CD8 TM protein sequence
IYIWAPLAGTCGVLLLSLVITLYC

SEQ ID NO: 14 - protein, 39 aa, Artificial Sequence
  CD28 hinge protein sequence
IEVMYPPPYLDNEKSNGTIIHVKGKHLCPSPLFPGPSKP

SEQ ID NO: 15 - protein, 39 aa, Artificial Sequence
  CD28 hinge protein sequence with C to S substitution
IEVMYPPPYLDNEKSNGTIIHVKGKHLSPSPLFPGPSKP

SEQ ID NO: 16 - protein, 27 aa, Artificial Sequence
  CD28 TM protein sequence
FWVLVVVGGVLACYSLLVTVAFIIFWV

SEQ ID NO: 17 - protein, 27 aa, Artificial Sequence
  CD28 TM with C to S substitution
FWVLVVVGGVLASYSLLVTVAFIIFWV

SEQ ID NO: 18 - protein, 41 aa, Artificial Sequence
  CD28 signalling domain protein sequence
RSKRSRLLHSDYMNMTPRRPGPTRKHYQPYAPPRDFAAYRS

SEQ ID NO: 19 - protein, 42 aa, Artificial Sequence
  4-1BB signalling domain protein sequence
KRGRKKLLYIFKQPFMRPVQTTQEEDGCSCRFPEEEEGGCEL

SEQ ID NO: 20 - protein, 112 aa, Artificial Sequence
  TCR zeta signalling domain protein sequence
RVKFSRSADAPAYQQGQNQLYNELNLGRREEYDVLDKRRGRDPEMGGKPRRKNPQEGLYNELQKDKMAEAYSEIGMKGERRRGKGHDGLYQGLSTATKDTYDALHMQALPPR

SEQ ID NO: 21 - protein, 22 aa, Artificial Sequence
  P2A protein sequence
GSGATNFSLLKQAGDVEENPGP

SEQ ID NO: 22 - protein, 9 aa, Artificial Sequence
  Synthetic peptide WT-1(37)
VLDFAPPGA

SEQ ID NO: 23 - protein, 9 aa, Artificial Sequence
  Synthetic peptide WT-1(126)
RMFPNAPYL

SEQ ID NO: 24 - protein, 9 aa, Artificial Sequence
  Synthetic peptide WT-1(187)
SLGEQQYSV

SEQ ID NO: 25 - protein, 9 aa, Artificial Sequence
  Synthetic peptide WT-1(235)
CMTWNQMNL